European Patent Application EP 4 303 308 A1, published January 10, 2024. Title: RECOMBINANT HOST CELLS PRODUCING IRONES AND USES THEREOF. Applicant: Museum National d'Histoire Naturelle. Application EP. The sequence listing filed with the application follows.

SEQUENCE LISTING (60 sequences)

SEQ ID NO: 1 - protein, 125 aa, Brevibacterium linens
MSAFEYLLLMGACLLITLPLELLFSARVYRRPKLLIGSLIPIILVFSLWDIIAIDRDHWTYNQQFVTGIHIGNLPLEELVFFIVIPICALLSYEAVGTVLKFVAKKSGTRAGRKSGNRKDGGDVA

SEQ ID NO: 2 - protein, 107 aa, Brevibacterium linens
MLPEYTVMTVVGIVIVIGLEIFVFRSGIFRRGQYWAALAICLAFQCLVDGWLTKLSDPIVRYNPSQFLNVRFPWDIPIEDFGFGFAMITSVLMLWQWQLNRSRKDTQ

SEQ ID NO: 3 - protein, 386 aa, Pantoe agglomerans
MPRYDLILVGAGLANGLIALRLRQQRPSLRILLIDAEREPGANHTWSFHAEDLTETQHRWIAPLVVHHWPGYEVRFPQRSRSMNSGYFCVTAERFAQVIRDRFAPDLLLNTRVASIASRAVTLDDGRVLESDAVIDGRGYQPDGALRMGFQSFVGQEWQLSEPHGLTAPIIMDATVDQQAGYRFVYSLPFSADTLLIEDTHYIDNATLEGDRARQNIHDYAAQQGWRLDRLLREEQGALPITLTGDVAAFWQNRDLPCSGLRAGLFHPTTGYSLPLAVALADRLAQMQTFTSETLHATIQQFASQAWQQQRFFRMLNRMLFLAGPADQRWQVMQRFYGLPEGLIARFYAGKLTLPDRLRILSGKPPVPVLAALQAIMTPHRQQAMQ

SEQ ID NO: 4 - protein, 585 aa, Porphyra umbilicalis
MAAFVSVPAGHLRPLRLSTAVSRRPLPGTAAAAPNGASPRAPRRRAAAAGIGMVTTPKPGSPSAAASPAPPSAAASVAAAAAAAVAAMPPTDSSQLYDVVVIGGGPAGLSLSAGLGERGLRTLVLDASLDTPWPNNYGVWLDELEALGLGDCTSAVWPDAVAYVRADGAPSALNRVYVRLDRHALKRRLLARCRASGAVTVVQAAAADVDVSPGTHSVVTYRDVAPATEGGADPDTPPGRPRMVGPVRSARGAVVADATGHALRFVEMEGAPAGGDGPSSLDLRGYQAAYGIEAVVEAHPYAPGQMVLMDYRDDHMQGSAAERTESATVPTFLYAMPTAPTRVFFEETSLIAAPAVPFEDLKRRLYARLAHDGITVTEVLDEEFCLIPMGGPLPVRQQRVVAFGGAAALVHPATGYMVARALELADEAAGHIAGELAAAKAKAAASLPAGGDPDGELEVDADAVASGVWEALWSVGRRKQRDFFNFGGEYLRRLDLPTIRDFFSAFFRLPRQQWAEFLSFRLLRPGERLAFGLGVFFRTTNRVRATITPFGMFHGRGKLLMSLLPLYPVDVPPPVKLPPLPEEGA

SEQ ID NO: 5 - protein, 411 aa, Synechococcus elongatus
MFDALVIGSGPAGLAIAAELAQRGLKVQGLSPVDPFHPWENTYGIWGPELDSLGLEHLFGHRWSNCVSYFGEAPVQHQYNYGLFDRAQLQQHWLRQCEQGGLQWQLGKAAAIAHDSHHSCVTTAAGQELQARLVVDTTGHQAAFIQRPHSDAIAYQAAYGIIGQFSQPPIEPHQFVLMDYRSDHLSPEERQLPPTFLYAMDLGNDVYFVEETSLAACPAIPYDRLKQRLYQRLATRGVTVQVIQHEEYCLFPMNLPLPDLTQSVVGFGGAASMVHPASGYMVGALLRRAPDLANAIAAGLNASSSLTTAELATQAWRGLWPTEKIRKHYIYQFGLEKLMRFSEAQLNHHFQTFFGLPKEQWYGFLTNTLSLPELIQAMLRLFAQAPNDVRWGLMEQQGRELQLFWQAIAAR

SEQ ID NO: 6 - protein, 673 aa, Phaffia rhodozyma
MTALAYYQIHLIYTLPILGLLGLLTSPILTKFDIYKISILVFIAFSATTPWDSWIIRNGAWTYPSAESGQGVFGTFLDVPYEEYAFFVIQTVITGLVYVLATRHLLPSLALPKTRSSALSLALKALIPLPIIYLFTAHPSPSPDPLVTDHYFYMRALSLLITPPTMLLAALSGEYAFDWKSGRAKSTIAAIMIPTVYLIWVDYVAVGQDSWSINDEKIVGWRLGGVLPIEEAMFFLLTNLMIVLGLSACDHTQALYLLHGRTIYGNKKMPSSFPLITPPVLSLFFSSRPYSSQPKRDLELAVKLLEEKSRSFFVASAGFPSEVRERLVGLYAFCRVTDDLIDSPEVSSNPHATIDMVSDFLTLLFGPPLHPSQPDKILSSPLLPPSHPSRPTGMYPLPPPPSLSPAELVQFLTERVPVQYHFAFRLLAKLQGLIPRYPLDELLRGYTTDLIFPLSTEAVQARKTPIETTADLLDYGLCVAGSVAELLVYVSWASAPSQVPATIEEREAVLVASREMGTALQLVNIARDIKGDATEGRFYLPLSFFGLRDESKLAIPTDWTEPRPQDFDKLLSLSPSSTLPSSNASESFRFEWKTYSLPLVAYAEDLAKHSYKGIDRLPTEVQAGMRAACASYLLIGREIKVVWKGDVGERRTVAGWRRVRKVLSVVMSGWEGQ

SEQ ID NO: 7 - protein, 427 aa, Prochlorococcus marinus
MPSKRLPDVLVLGAGPAGMAIASALGKEKLEVEVLSPNGPDEPWPNTYGIWGKEVDQLGLQDLLEYRWKNTVSFFGHGSLEEHHYENKATEHSLDYGLFDKKKLHRYWLNECNKSLIKWHEGFAEKITFQKHKSTVITSNGKTYSARLVVDATGYDPVFLKLKSCGPLAVQTCYGIVGSFSKPPLKKGQFVLMDYRNDHLNEEQKKEPPTFLYAMDMGNGKYFLEETSLGLVNPLTMEDLKERLEKRLSYRNISITSMQHEELGLFLPMNMPIPDFKQQVLGYGGAASMVHPASGYLIGNVLRRAPLVAKAISTAMNDKKLSTYHIARKGWESLWPKELIRKKSIYQFGLEKLMRFDEKLLREFFGSFFKLPKTQWYGFLTDTLSLREIVYAMCIMFIRAPWSVKKGLMIMHGKELRMLLRIVLPNI

SEQ ID NO: 8 - protein, 424 aa, Vulcanococcus limneticus
MAVDVLVIGSGPAALAIAAALVEQGLMVEALASVDPEVPWANTYGIWGPEVDALGLEALLGHRWSHTSSYFGADPQSPATEHGTGQRGAVSHGIDYGLFDKTKLQHHWLEQCRGGGLRWHRGLATAIRHEALQSTVTTQEGQELSARLVVDASGHQPVFVQRPDDGPVAGQAAYGVVGTFSAPPVQPGQFVLMDYRCDHLTPQERWESPTFLYAMDLGGGVFFVEETSLALAPPVPYDTLKDRLLRRLAHRGVQVLEIQHEEFCLFPMNLPLPDLGQQVVGFGGAASMVHPASGYMVGALLRRAPVLAAAIASGLRTPGLDSANLARRAWAALWPLQLRRKHALYRFGLDKLMRFPEAQLRAFFANFFAMPPAQWYGFLTNTLPLPQLIAAMLRLFATAPWSVRWGLLEPRGRELALLGRLFWP

SEQ ID NO: 9 - protein, 417 aa, Synechococcus sp. BS55DK
MAEPVDVLVLGGGPAALCIASELNQRGVAVAAIAPDPVDAPWPNTYGIWADELKAVGLEHLLEHRWSDTVSYFGDGGSTAQDQSHAHGIDYGLFDRAALQRYWLERADGVVWHQDTAQRLEVNGATTSVSCVSGTMLQARLVIDASGSRTPHIRRPDQGPVAGQAAYGVVGRFSKPPIEAGRFVLMDYRCDHLSEVQRHEPPTFLYAMDLGDGVFFVEETSLALAPGVPYDVLKQRLQQRLDLRGVEIIEVIHEEFCLFPMNLPLPDRSQPVLAFGGAASMVHPASGYMVGSLLRRGPDLAQAISEALANPSLGSAALSQRGWQSLWPIELVLRHQLYQYGLGRLMGFNEALLRTHFSTFFSLPREEWFGFLTNTLSLPRLMAVMLRLFVLSPWELRRGLVLGAGTHQRPTFLQSAG

SEQ ID NO: 10 - protein, 422 aa, Cyanobium sp. CACIAM 14
MLVIGSGPAALTIAAELGERGVAVEALSATEPEAPWPNTYGIWGDEVDALGLGHLLAHRWTDTVSYFGAGCEQGSEPTPHGRDYGLFDKQALQSHGLERCAAAGLRWHRGRADGIEHGEDGSTVHTEAGERRHARLVIDATGHEPCFVTRPSDGPVAGQAAYGIVGRFSAPPVEPGRFVLMDYRCDHLRPEELAEPPTFLYAMDLGDGRFFVEETSLALAPPVPFAVLQDRLQRRLARRGAAVTTIEHEEFCLFPMNPALPDPAQRVVGFGGAASMVHPASGYLVGGLLRRAPALAAAISTALGAPELDGAALAAAAWEGLWPADLRRKHALYRFGLEKLMRFREDQLRHFFRTFFRMPNAQWYGFLTNTLTVPETFRAMLGLFARAPNDVRWGLMAPEGRELALLAKVLDPDAAVFRASPG

SEQ ID NO: 11 - protein, 427 aa, Prochlorococcus sp. HOT208
MSKENMPDVLVLGAGPAGMAIASALGKEKLDVEVLSPNGPDEPWPNTYGIWGKEVDQLGLQDLLEYRWKNTVSFFGHGALEEQDDENKATEHSLDYGLFDKKKLHNYWFNECNKSFIKWHQGFANKIHFEKYKSTVTTKDGKNYSARLVVDATGYDPVFLKLKSCGPLAVQTCYGIVGNFSKPPLKEGQFVLMDYRNDHLNDAQKKEPPTFLYAMDMGGGKYFLEETSLGLVNPLTMENLKERLEKRLSYRNISITSMQHEELGLFLPMNMPIPDFKQQILGYGGAASMVHPASGYLIGNVLRRAPLVAKAVSEAIKHKNLSTYHIARRGWETLWSKELIRKKSLYQFGLEKLMRFDEKLLREFFGSFFQLPKNQWYGFLTDTLSLKEIVYAMCVMFIKAPWSVKKGLMIMHGREFKMLLRIIFPNI

SEQ ID NO: 12 - protein, 491 aa, Porphyra umbilicalis
APAAQPGAAPPRTYDVTVIGGGPAGLSLAAALSATGVTVAVLDAKIDVPWPNHYGVWADEFEPLGLGDCATSTYPRTTIYVPDGPGGGPVVLNRRYLRVDRVKLKARLLERCAAGGVVIEPAHVSAVEHVSATHSTVTFVEGDGVGGGGGGGGGDGGRPPASQQLRTRLVVDATGHALRFVQTSPGYSPGFQAAYGIEAVVESHPFPVDEMLLMDFRDDHMQGDAADAATSSAAPTFLYVFPTDEKRVFLEETSIIAPTAVPFEALRERLYKRLDHLGVTVTSVTEEEYSLIPLGGVVPLLGQRVVGFGGSACLVHPATGYMVARTLSLAESLAAEIATALRAPPTAAAAAPSGQRGDGGGAPPLAPSDAVAAAAWAHLWSESRIRERDFLLFGADLLAGLDLGAMKEFFAAFFRLPQPLWAGFLSFRLAAPSERATFAFVFFLQASNRIRAGLLRGIVTIGRWKLIGGVVPLWLARIGDGAGEEQRRGGE

SEQ ID NO: 13 - protein, 540 aa, Oryza sativa
MEFSGGATVSAPFGCCRAAWGAAAAGAGAEGRSRRVVPRAVEPRRRGRWMVRCVATEKHKDAAARRGGVEVEFADEEDYVKGGGGELLYVQMQASKSMDSQSKISSKLLPIPDENSVLDLVIIGCGPAGLSLAAESAKKGLNVGLIGPDLPFTNNYGVWEDEFKDLGLESCIEHVWKDTIVYLDGNKPIMIGRAYGRVHRDLLHEELLRRCYDAGVTYLSSKVDKIMESPDGHRVVCCEGDREVLCRLAIVASGAASGRLLEYEVGGPRVCVQTAYGVEVEVENNPYDPSLMVFMDYRDCFKDKFSHPEQGNPTFLYAMPMSSTRIFFEETCLASKEAMPFDLLKKRLMSRLDAMGVHIRKVYEEEWSYIPVGGSLPNTDQKNLAFGAAASMVHPATGYSVVRSLSEAPRYASVISDILRNRVYPGEYLPGTSQSSSPSMLAWRTLWPQERKRQRSFFLFGLALIIQLNNEGIQTFFETFFRLPKWMWRGFLGSTLSSVDLILFAFYMFTIAPNQMRMNLVRHLLSDPTGSTMIKTYLTL

SEQ ID NO: 14 - protein, 537 aa, Zea mays
MGLSGATISAPLGCCVLRCGAVGGGKALKADAERWRRAGWSRRVGGPKVRCVATEKHDETAAVGAAVGVDFADEEDYRKGGGGELLYVQMQSTKPMESQSKIASKLSPISDENTVLDLVIIGCGPAGLSLASESAKKGLTVGLIGPDLPFTNNYGVWEDEFKDLGLESCIEHVWKDTIVYLDNNKPILIGRSYGRVHRDLLHEELLKRCYEAGVTYLNSKVDKIIESPDGHRVVCCDKGREIICRLAIVASGAASGRLLEYEVGGPRVCVQTAYGVEVEVENNPYDPSLMVFMDYRDCFKEEFSHTEQENPTFLYAMPMSPTRVFFEETCLASKDAMSFDLLKKRLMYRLNAMGIRILKVYEEEWSYIPVGGSLPNTDQKNLAFGAAASMVHPATGYSVVRSLSEAPRYASVISDILGNRVPAEYMLGNSQNYSPSMLAWRTLWPQERKRQRSFFLFGLALIIQLNNEGIQTFFEAFFRVPRWMWRGFLGSTLSSVDLILFSFYMFAIAPNQLRMNLVRHLLSDPTGSSMIKTYLTL

SEQ ID NO: 15 - protein, 654 aa, Chromochloris zofingiensis
MGTPAATVVLAFGWHVEFASAYYSHLSWLICWHVLGPTARPIAYEPQTSHYNHSQSCLRRLLAVASLRLAWVVPTWCCISRANSMQPALVDRPAARCSCLGRQYHTKPFTSHPRTQPARQARSNVSVAYPIDAVTTPSPGGGHDHNQAVREGHYEADLVKAQANKQDGEQPKIASILQPLQVGTKADAVVVGCGPAGLYLAAQMAQRGLKVGLIGPDVPFVNNYGVWVDEFKQLGLEHTLECQWPDAVCYFGEGNQVNVGRAYGRVCRRRLRQHLVDLCKSAGVQYLATEVTDICKSADNTTAYVTCSNGSTFTSRLVTLASGQAAGRFLQYEPEAPAVAAQTAYGIEAEVEGYDAAYGNDHMLFMDYRRHHTGLWDGGATKLNAGNHPNANDGLWGSSDEVPSFLYAMPLGGNRVFLEETCLVAKPALPFKVLQRRLERRMRSMGIKVTRIHETEWSYIPVGGPLPSANQPITAFGAAANLVHPATGFSVSRSLREAPVMAEAAVQALSGSQTVPEVAAAVWQALWPDEKRRQASFHLFGMELLAQLDLSATNAFFNTFFALPPTYWKGFLGSRLSSVQLLGFALLTFVLAPANIKGKLVSHLMTDPAGRYLISHYISGWSSKESAMTGAPTEAAVAAALMMWQLAAATQVQQ

SEQ ID NO: 16 - protein, 575 aa, Haematococcus lacustris
MAAAQGSLTTRQCLAASRSSAAPTRLQPLRVATVARPIVESPTSPQDSHLRIPVVQDQNQLVRVGHYEAALVRQQASKPDSGQDAIASSLHKPDMSKLHDAVVVGAGPAGMYLAAELAKRGLSTVLVGLDMPLVNNYGVWTDEFKALGLEHTLERSWPDASCFFGEGKPVRLGRGYGRVSRRKLREHLVAMCAEAGVAFLAAEVDSLQVAVGGGSTTLSMLHGGQLRARLVTLAAGAAAGKFLRYEEGAPSVASQTAYGIEAEVEGYHEAFPGNEMLFMDFRRHHTGVWEQSAPKIRVGSHPNAGDGEWGTSGEVPSFLYAMPLGGDRVFLEETCLVAKPALPFAVLKRRLERRMAAHGIRVKKVHEEEWSYIPVGGPLPKGDQAVAAFGAAANLVHPATGFSVSRSFREAPRVADELAACIRAGLGVRQASARVWSTLWPQEKRTQTAFHVFGMELLATLDLASTNAFFGTFFKLPSYYWRGYMASQLSSGELIIFALLTFTLANNDIRAKLMVHLFSDPAGRYLLDAYVKRYRDSPSPSPSSSPSSSLSALPPPAPAPAAEVKLPASLEPNQA

SEQ ID NO: 17 - protein, 303 aa, Streptomyces niveus
MSNLDELSSPPQTVLESQDEVGIVGQYYDDKTARLVRKYGPGPRIHYHVGHYPSSQTPLNVQEATADAIRGSIRIHQEGLLRYAAKIWGAEHRLSGRILDVGCGLGGGSLFWAQEYGADVTAVTNAPEHAPIVEGFARECGVGGQVRALVCDAMHLPLDDGPYDAAVAIESSGYFDRPQWFERLARVLRPGGSVCIEEVFTTRPHGADVWAEYFYTKPASVLDYAEAAKAAGFELVDDVDATSETQPFWEESAAWTKAVLDSDDTLSAVARRQLRISLLANQALGTEWKAGGLRLGFLRFELR

SEQ ID NO: 18 - protein, 303 aa, Streptomyces sp. RI18
MSNLDELASSRQTVLEPQDEVRIVGQYYDDKTAKLVRKYGPGPRIHYHVGYYPSSEAPRHTRDVTPDAFRRSIRLHQEGLLRYAAKIWGAEHRLSGRILDVGCGLGGGSLFWAQEYGADVTAVTNAPEHAPIVEGFARECGVGGRVRTLVCDAMHLPLDGGPYDAAVAIESSGYFDRPVWFERLAHVLRPGGSVCIEEVFTTRPHGADVWAEYFYTKPATVLDYAEAAKAAGFELVDDVDATSETLPFWEESTAWTKAVLDSDSTLSAVDRRQLRISLMANQALGAEWQAGGLRLGFLRFERK

SEQ ID NO: 19 - protein, 303 aa, Streptomyces sp. 4R-3d
MSNLDELSSPPQTALESQDEVGIVGQYYDDKTARLVRKYGPGPRIHYHVGHYPSSQTPLNVQEATADAIRGSIRIHQEGLLRYAAKIWGAEHRLSGRILDVGCGLGGGSLFWAQEYGADVTAVTNAPEHAPIVEGFARECGVGGQVRALVCDAMHLPLDDGPYDAAVAIESSGYFDRPRWFERLSRVLRPGGSVCVEEVFTTRPHGADVWAEYFYTKPASVLDYAEAAKAAGFELVDDVDATSETQPFWEESAAWTKAVLDSDDTLSAVARRQLRISLLANQALGTEWQAGGLRLGFLRFELR

SEQ ID NO: 20 - protein, 302 aa, Streptomyces ipomoeae
MSNLDGLSSSPHAALEPQDEVRIVGQYYDDKTARLIRKYGPGPRIHYHVGYYPSSETPLNAQDATPDAIRRSIRLHQEGLLRYAAKIWGAEHRLSGRILDVGCGLGGGSLFWAQEYGADVTAVTNAPEHAPIVDGFARECGVDGKVRTLVCDAMHLPLDGPYDAAVAIESSGYFNRPLWFERLARVLRPGGSVCIEEVFITRPHGADVWAEYFYTKPATVLDYAEAAKSAGFELVDEVDATSETLPFWEESAAWTKAVLDSDSSLSAVDRRQLRISLMANQALGAEWQAGGLRLGFLRFELK

SEQ ID NO: 21 - protein, 304 aa, Streptomyces malaysiensis
MSNLDELSGSPQTVLEPQDEVKVVGQYYDDKTARLVRKYGPGPRIHYHVGHYPSSKSPLDAHDATPDAIRGSIRTHQEGLLRYAAKIWGAEHRLSGRILDVGCGLGGGSIFWAQEYGADVTAVTNAQEHAPIVEGFARECGLDGKVRALVSDAMHLPLDGGPYDAAVAIESSGYFNRPQWFERLSHVLRPGGSVCIEEVFITRPHGADVWAEYFYTKPATVRDYTEAAQAAGFELVDDVDATSETLPFWEESAAWTKAVLDSDDSLSPVDRRNLRISLLANEALGAEWGAGGVRLGFLRFELKK

SEQ ID NO: 22 - protein, 303 aa, Streptomyces sp.
MSNLDELSGSPQTVLEPQDEVKVVGQYYDDKTARLVRKYGPGPRIHYHVGHYPSSKSPLDAHDATPDAIRGSIRTHQEGLLRYAAKIWGAEHRLSGRILDVGCGLGGGSIFWAQEYGADVTAVTNAQEHAPIVEGFARECGLDGKVRALVSDAMHLPLDGGPYDAAVAIESSGYFNRPQWFERLSHVIRPGGSVCIEEVFITRPHGADVWAEYFYTKPATVRDYTEAAQAAGFELVDDVDATSETLPFWEESAAWTKAVLDSDDSLSPVDRRNLRISLLANEALGAEWGAGGVRLGFLRFEKK

SEQ ID NO: 23 - protein, 301 aa, Streptomyces antimycoticus
MSNLDELSGSPQTALEPQDEVKVVGQYYDDKTARLVRKYGPGPRIHYHVGHYPASQSPLDAHDATPDAIRGSIRTHQEGLLRYAAKIWGAEHRLSGRILDVGCGLGGGSLFWAQEYGADVTAVTNAQEHAPIVDGFARECGLDGKVRALVSDAMHLPLDGGPYDAAVAIESSGYFNRPQWFERLSHVLRPGGSVCIEEVFITRPHGADVWAEYFYTKPATVLDYTEAAQAAGFELVDDVDATSETLPFWEESAAWTKAVLDSDSSLSPVDRRNLRISLLANEALGAEWGAGACGWASCASS

SEQ ID NO: 24 - protein, 304 aa, Streptomyces antioxidans
MSNLDELSSSPQTALEPQDEVKIVGQYYDDKTARLVRKYGPGPRIHYHVGHYPSSVAPPHADDATPDAIRGSIRSHQEGLLRYAAKIWGAEHRLSGKILDVGCGLGGGSLFWAQEYGADVTAVTNAQEHAPIVEGFARECGVDGKVRALVSDAMQLPLDGGPYDAAVAIESSGYFNRPQWFERLAHVLRPGGSVCVEEVFITRPHGADVWAEYFYTKPATVRDYAEAAQAAGFELVDDVDATSETLPFWEESAAWTKAVLDTDSSLSPVDRRNLRISLLANQALGAEWGAGGLKLGFLRFELKK

SEQ ID NO: 25 - protein, 302 aa, Streptomyces sp. 150FB
MSNLDELSSSRQTVLEPEDEVRIVGQYYDDKTARLVRKYGPGPRIHYHVGHYPSSETPLHEDDATPDAIRQSIRSHQEGLLRYAAKLWGAEHRLSGRILDVGCGLGGGSLFWAQEYGADVTAVTNAPEHAPIVDGFARECGLEEKVRARVSDAMHLPLDGPYDAAVAIESSGYFNRPQWFERLSRVLRPGGSVCIEEVFTTRPHGADVWAEYFYTKPATVLDYVEAAQAAGFELVDDVDATSETAPFWDESAAWTKAVLDTDSSLSAVARRQLRISLMANQAVGAEWRAGGLRLGFLRFELK

SEQ ID NO: 26 - protein, 304 aa, Streptomyces caeruleatus
MAVSNLDELSSSSQKVLEHQDETRLVGQYYDDKTARLVRKYGPGPRIHYHVGHYPSSRTPVDVHEATPDDIRRSIRLHQEGLLRYAAKIWGAEHRLSGRILDVGCGLGGGSLFWAQEYGADVTAVTNAPEHAPIVERFAQESGVGEKVRTLVCDAMHLPLDGPYDAAVAIESSGYFNRPQWFERLARVIRPGGSVCIEEVFITRPHGADVWSEYFYTKPATVRDYAEAARAAGFELVDDVDATSETAPFWEESTAWTKAVLDSDNSLSAVERRQLRISLMANQALGAEWRAGGLRLGFLRFELK

SEQ ID NO: 27 - protein, 315 aa, Streptomyces adelaidensis
MDGLSSSAQTVLEPQNEVRIVGQYYDDKTARLVRKYGPGPRIHYHVGHYPSSRTPLNVHEATPDDLRGSIRLHQEGLLRYAAKIWGAEHRLSGRILDVGCGLGGGSLFWAQEYGADVTSITNAPEHAPIVEGFARESGVGGKIRTLVCDAMHLPLDDGPYDAAVAIESSGYFDRPQWFERLGHVIRPGGSVCIEEVFITRPHGADVWAEYFYTKPATVRDYAEAAEAAGFELVDDVDATSETLPFWEESTAWTKAVLDGDSSLSPVERRQLRISLLANQALGAEWAAGGLRLGFLRFERKRAASIPADSPGPRGT

SEQ ID NO: 28 - protein, 303 aa, Streptomyces kasugaensis
MSNLDELSSSPQAALDPQDEVKIVGQYYDDKTAKLVRKYGPGPRIHYHVGYYPSFEAPPRADDVTPDDIRGSIRRHQEDLLRYAAKIWDAEQRLSGRVLDVGCGLGGGSLFWAEEYGADVTAVTNAPEHAPVVEGFARECGVGGRVRALVSDAKQLPLDSGPYDAAVAIESSGYFDRPLWFERLAQVLRPGASVCIEELFITRPHGADVWAEYFYTKPATVLDYVKAAEAAGFELVDDVDATAATAPFWEESVAWTEAVLDSDSGLSPVDRRQLRISLLANRALGAEWQAGGARLGFLRFELK

SEQ ID NO: 29 - protein, 303 aa, Streptomyces acidiscabies
MSDLDELSGSAQQVLEPQDEVRIVGQYYDEKTAKLVRKYGPGPRIHYHVGHYPSSRTPLDVHDATADDIRHSIRIHQEGLLRYAAKIWGAEHRLSGRVLDVGCGLGGGSLFWAQEYGADVTSVTNAPEHAPVVEGFAQEAGVGGRVRALVCDAMHLPQDGGPYDAAVAIESSGYFDRPRWFDRLSNIIRPGGSVCIEEVFITRPHGADVWAEYFYTKPTTVRAYAEAAEAAGFELVDDVDATPETAPFWDESTAWTKAVLDSDDSLSSVERRQMRISLMANQALGTEWRAGGLKLGFLRFERK

SEQ ID NO: 30 - protein, 324 aa, Lentzea indica
MHNDHIRPFTKVVGIRGPGEVTVSNLDEISSPPQTAPDLQDESRMVGQYYDDKTAKLVRKYGPGPRIHYHVGYYPASETPPHAHDATPEAIRHSIRLHQEGLLRYAAKIWGAEHRLSGRILDVGCGLGGGSLFWAQEYGADVTAITNAPEHPPIVDGFARECGVDGKVRTLVRDATQLPLDGPYDAAVAIESSGYFNRPLWFERLARVLRPGGSVCIEEVFITRPHGADVWAEYFYTKPVTVLDYVEAAKSAGFELVDDVDATSETSPFWDESAAWTKAVLDSDSSLSAVARRQMRISLLANQALGTEWKAGGLKLGFLRFELK

SEQ ID NO: 31 - protein, 302 aa, Saccharothrix espanaensis
MSDLDELSSPPQAVLDPPDEVGLVGQYYDDKTARLVRKYGPGPKIHYHVGYYPSAERPLRAHDATPDAIRRSIRCHQEGLLRYAAEVWDAGHRLSGKVLDVGCGLGGGSIFWAQEYGADVTAVTNAPEHAPIVDGFARECGLGRQVRTLVCDAMQLPVSGPYDAAVAIESSGYFHRARWFERLARVLRPGGNVCVEEVFLTRPHGADVWAEYFYTRPATVLDYAQAARSAGFELVDEVDATSETLPFWEESTAWTKAVLDSDSSLSAVDRRQLRISLMANQALGAEWRAGGLRLGFLRFELR

SEQ ID NO: 32 - protein, 299 aa, Escherichia coli
MDFPQQLEACVKQANQALSRFIAPLPFQNTPVVETMQYGALLGGKRLRPFLVYATGHMFGVSTNTLDAPAAAVECIHAYSLIHDDLPAMDDDDLRRGLPTCHVKFGEANAILAGDALQTLAFSILSDADMPEVSDRDRISMISELASASGIAGMCGGQALDLDAEGKHVPLDALERIHRHKTGALIRAAVRLGALSAGDKGRRALPVLDKYAESIGLAFQVQDDILDVVGDTATLGKRQGADQQLGKSTYPALLGLEQARKKARDLIDDARQSLKQLAEQSLDTSALEALADYIIQRNK

SEQ ID NO: 33 - protein, 296 aa, Bacillus subtilis
MTNKLTSFLADRKKTIENQLSVYTEKLDMPDSLKKSMLYSLQAGGKRLRPLIVLAVLNAYGKSEKDGIPVGCAVEMIHTYSLIHDDLPCMDDDDLRRGKPTNHKVFGEATAVLAGDGLLTESFKLITSHVSDEVSAEKRLRLVNELISAAGTEGMVGGQVADMEAENRQVTLEELESIHERKTAKLLGFCVIAGAILADAPEEDIETLRTFSSHIGIGFQIRDDILDLEGSEEKIGKRVGSDTTNDKSTYPSLLSLEGAKHKLDVHIKEAKRLIGGLSLQKDLLYELCDLIAARDH

SEQ ID NO: 34 - protein, 299 aa, Pantoea agglomerans
MDFANELQARVVRANDALRRFIAPQPFQNTPLVEAMQYGALLGGKRLRPFLVYATGNMFGISDNTLDAPAAAVECIHAYSLIHDDLPAMDDDDLRRGQPTCHIKFGEANAILAGDALQTLAFSILSDAPMAEVADRDRLAMISELAMASGVAGMCGGQALDLEAEGRQVNLEQLERIHRHKTGALIRSAVRLGALSAGEQGRKALPTLDRYAESIGLAFQVQDDILDVVGDTATLGKRQGADQQLGKSTYPALLGLEQAQRKARDLIDDARQSLNVLAAQSLDTSALEALADYIIQRDK

SEQ ID NO: 35 - protein, 352 aa, Saccharomyces cerevisiae
MASEKEIRRERFLNVFPKLVEELNASLLAYGMPKEACDWYAHSLNYNTPGGKLNRGLSVVDTYAILSNKTVEQLGQEEYEKVAILGWCIELLQAYFLVADDMMDKSITRRGQPCWYKVPEVGEIAINDAFMLEAAIYKLLKSHFRNEKYYIDITELFHEVTFQTELGQLMDLITAPEDKVDLSKFSLKKHSFIVTFKTAYYSFYLPVALAMYVAGITDEKDLKQARDVLIPLGEYFQIQDDYLDCFGTPEQIGKIGTDIQDNKCSWVINKALELASAEQRKTLDENYGKKDSVAEAKCKKIFNDLKIEQLYHEYEESIAKDLKAKISQVDESRGFKADVLTAFLNKVYKRSK

SEQ ID NO: 36 - protein, 297 aa, Geobacillus stearothermophilus [sequence omitted]

SEQ ID NO: 37 - protein, 367 aa, Gallus gallus
MHKFTGVNAKFQQPALRNLSPVVVEREREEFVGFFPQIVRDLTEDGIGHPEVGDAVARLKEVLQYNAPGGKCNRGLTVVAAYRELSGPGQKDAESLRCALAVGWCIELFQAFFLVADDIMDQSLTRRGQLCWYKKEGVGLDAINDSFLLESSVYRVLKKYCRQRPYYVHLLELFLQTAYQTELGQMLDLITAPVSKVDLSHFSEERYKAIVKYKTAFYSFYLPVAAAMYMVGIDSKEEHENAKAILLEMGEYFQIQDDYLDCFGDPALTGKVGTDIQDNKCSWLVVQCLQRVTPEQRQLLEDNYGRKEPEKVAKVKELYEAVGMRAAFQQYEESSYRRLQELIEKHSNRLPKEIFLGLAQKIYKRQK

SEQ ID NO: 38 - protein, 346 aa, Artemisia tridentata
MSSSKSIDLKSKFLKVYDTLKSDLINDPAFEFDDDSRQWIQKMLDYNVPGGKLNRGLSVVDSYQLLKGGELSDDEIFLSSALGWCIEWLQAYFLVLDDIMDESHTRRGQPCWFRLPKVGMIAANDGILLRNHVPRILKKHFRGKPYYVDLVDLFNEVEFQTASGQMIDLITTLVGEKDLSKYSLSIHRRIVQYKTAYYSFYLPVACALLMFGEDLDKHVEVKNVLVEMGTYFQVQDDYLDCFGAPEVIGKIGTDIEDFKCSWLVVKALELANEEQKKTLHENYGKKDPASVAKVKEVYHTLNLQAVFEDYEATSYKKLITSIENHPSKAVQAVLKSFLGKIYKRQK

SEQ ID NO: 39 - protein, 302 aa, Pantoea agglomerans
MTVCAEQHVNFIHSDAASLLNDIEQRLDQLLPVESERDLVGAAMRDGALAPGKRIRPLLLLLAARDLGCNATSAGLLDLACAVEMVHAASLILDDMPCMDDAQLRRGRPTIHCQYGEHVAILAAVALLSKAFGVVAAAEGLTATARADAVAELSHAVGMQGLVQGQFKDLSEGDKPRSADAILMTNHYKTSTLFCASMQMASIVAEASGEAREQLHRFSLNLGQAFQLLDDLTDGMADTGKDAHQDDGKSTLVNLLGPQAVETRLRDHLRCASEHLLSACQDGYATHHFVQAWFEKKLAAVS

SEQ ID NO: 40 - protein, 335 aa, Saccharomyces cerevisiae [sequence omitted]

SEQ ID NO: 41 - protein, 329 aa, Deinococcus radiodurans
MRPELLARVLSLLPETSATPELARFYALLRDYPQRGGKGIRSELLLASARAHGLSESDTGWESALWLAAALELFQNWVLVHDDIEDDSEERRGRPALHHLCGMPVALNVGDALHAYMWAAVGKANVPGAFEEFLQMVYRTAEGQHLDLAWVEGREWGLRPADYLQMVGLKTAHYTVIVPLRLGALAAGMAPQDAFTPAGLALGTAFQIRDDVLNLAGDPVKYGKEIGGDLLEGKRTLIVLDWLTTAPDDRKAIFLDQMRRHRADKDPAVIDEIHRWLLESGSVEAAQDYAQAQAAEGLDLLEKALADAPDAQAAAALLASVRELATREK

SEQ ID NO: 42 - protein, 302 aa, Synechococcus sp.
MVVADAHTQGFSLAQYLQEQKTIVETALDQSLVITEPVTIYEAMRYSLLAGGKRLRPILCLAACEMLGGTAAMAMNTACALEMIHTMSLIHDDLPAMDNDDLRRGKPTNHKVYGEDIAILAGDALLSYAFEYVARTPDVPAERLLQVIVRLGQAVGAEGLVGGQVVDLESEGKTDVAVETLNFIHTHKTGALLEVCVTAGAILAGAKPEEVQLLSRYAQNIGLAFQIVDDILDITATAEELGKTAGKDLEAQKVTYPSLWGIEKSQAEAQKLVAEAIASLEPYGEKANPLKALAEYIVNRKN

SEQ ID NO: 43 - protein, 289 aa, Rhodobacter capsulatus
MSLDKRIESALVKALSPEALGESPPLLAAALPYGVFPGGARIRPTILVSVALACGDDCPAVTDAAAVALELMHCASLVHDDLPAFDNADIRRGKPSLHKAYNEPLAVLAGDSLLIRGFEVLADVGAVNPDRALKLISKLGQLSGARGGICAGQAWESESKVDLAAYHQAKTGALFIAATQMGAIAAGYEAEPWFDLGMRIGSAFQIADDLKDALMSAEAMGKPAGQDIANERPNAVKTMGIEGARKHLQDVLAGAIASIPSCPGEAKLAQMVQLYAHKIMDIPASAERG

SEQ ID NO: 44 - protein, 325 aa, Methanobacterium thermoautotrophicum
MMEVMDILRKYSEMADERIRESISDITPETLLRASEHLITAGGKKIRPSLALLSSEAVGGDPGDAAGVAAAIELIHTFSLIHDDIMDDDEIRRGEPAVHVLWGEPMAILAGDVLFSKAFEAVIRNGDSEMVKEALAVVVDSCVKICEGQALDMGFEERLDVTEEEYMEMIYKKTAALIAAATKAGAIMGGGSPQEIAALEDYGRCIGLAFQIHDDYLDVVSDEESLGKPVGSDIAEGKMTLMVVKALERASEKDRERLISILGSGDEKLVAEAIEIFERYGATEYAHAVALDHVRMAKERLEVLEESDAREALAMIADFVLEREH

SEQ ID NO: 45 - protein, 340 aa, Pyrococcus furiosus
MYDELFKKIKEKAKFVDEKLLSLIPEKEPKILYEAARHYPLAGGKRVRPFVVLTATEAVGGEWEKAIYPAVAIELIHNYSLVHDDIMDMDETRRGRPTVHKVWGINMAILAGDLLFSKAFEAISRAEIPPEKKARVLETVVKASNELCEGQAMDLEFEKRDTVTIEEYMRMISGKTGALFDASAKVGGIVGTDNEEYINALSTWGRNVGIAFQIWDDVLDLIADEEKLGKPVGSDIRKGKKTLIVAHFFENADEKDKQKFLKVFGKYAGDVKGEGIIEEDIKAEVMEAIDLLKKYGSIDYAANIAREMVKKANEALKVLPESEARKDLELLARFIVEREY

SEQ ID NO: 46 - protein, 295 aa, Pantoea agglomerans
MEVGSKSFATASKLFDAKTRRSVLMLYAWCRHCDDVIDDQVLGFSNDTPSLQSAEQRLAQLEMKTRQPMRIQMHEPAFAAFQEVAMAHDILPAYAFDHLAGFAMDVHETRYQTLDDTLRYCYHVAGVVGLMMAQIMGVRDNATLDRACDLGLAFQLTNIARDIVEDAEAGRCYLPAAWLAEEGLTRENLADPQNRKALSRVARRLVETAEPYYRSASAGLPGLPLRSAWAIATAQQVYRKIGMKVVQAGSQAWEQRQSTSTPEKLALLVAASGQAVTSRVARHAPRSADLWQRPV

SEQ ID NO: 47 - protein, 339 aa, Rhodobacter capsulatus
MIAEADMEVCRELIRTGSYSFHAASRVLPARVRDPALALYAFCRVADDEVDEVGAPRDKAAAVLKLGDRLEDIYAGRPRNAPSDRAFAAVVEEFEMPRELPEALLEGFAWDAEGRWYHTLSDVQAYSARVAAAVGAMMCVLMRVRNPDALARACDLGLAMQMSNIARDVGEDARAGRLFLPTDWMVEEGIDPQAFLADPQPTKGIRRVTERLLNRADRLYWRAATGVRLLPFDCRPGIMAAGKIYAAIGAEVAKAKYDNITRRAHTTKGRKLWLVANSAMSATATSMLPLSPRVHAKPEPEVAHLVDAAAHRNLHPERSEVLISALMALKARDRGLAMD

SEQ ID NO: 48 - protein, 492 aa, Pantoea agglomerans
MNRTTVIGAGFGGLALAIRLQASGVPTRLLEQRDKPGGRAYVYQDQGFTFDAGPTVITDPSAIEELFTLAGKKLSDYVELMPVKPFYRLCWESGKVFSYDNDQPALEAQIAAFNPRDVEGYRRFLAYSRAVFAEGYLKLGTVPFLSFRDMLRAAPQLAKLQAWRSVYSKVASYIEDEHLRQAFSFHSLLVGGNPFATSSIYTLIHALEREWGVWFPRGGTGALVQGMVKLFEDLGGEVELNASVARLETQENRITAVHLKDGRVFPTRAVASNADVVHTYRELLSQHPASQAQGRSLQNKRMSNSLFVIYFGLNHHHDQLAHHTVCFGPRYRELIDEIFNKDGLAEDFSLYLHAPCVTDPSLAPEGCGSYYVLAPVPHLGTADIDWAVEGPRLRDRIFDYLEQHYMPGLRSQLVTHRIFTPFDFRDELNAYQGSAFSVEPILTQSAWFRPHNRDKNINNLYLVGAGTHPGAGIPGVIGSAKATAGLMLEDLA

SEQ ID NO: 49 - protein, 494 aa, Rhodobacter capsulatus
MRSETDVVVIGAGMGGLAAAIGAAAAGLRVTVVEAGDAPGGKARAVATPGGPADTGPTVLTMRHVLDALFAACGTRTDEHLTLIPLPRLARHFWPDGASLDLFTDTEANIEAIRAFAGDKEAAAFRRFDHLSAGLWDAFHRSVIAAPKPDLLRIAAATATHPPLWPALRPGLTMRDLLAHHFKDPRLAQLFGRYATYVGGRPGATPAVLSLIWQAEVQGVWAIREGMHGVAAALARVAEAKGVRFHYGAKAKRIVRKEGRVTAVEIETGASIPCGACIFNGDPGALRDGLLGDAARASMEKTARPAPSLSAWVWAFGATPRGVDLAHHNVFFTADPELEFGPIGAGEMPEEPTLYICAQDREMQAPVPEIERFEIIMNGPAGHQPFPQEEAQCRARTFPMLAAMGLTFSPDPETRALTTPALLSRRFPGSLGAIYGGSPEGTLATFRRPLARTGLKGLYLAGGGTHPGAGVPMALTSGTHAARALLADRISAAK

SEQ ID NO: 50 - protein, 543 aa, Osmanthus fragrans
MGMQGEDAQRTGNIVAVKPKPSQGLTSKAIDWLEWLFVKMMHDSKQPLHYLSGNFAPVDETPPLKDLPVTGHLPECLNGEFVRVGPNPKFASIAGYHWFDGDGMIHGMRIKDGKATYVSRYVQTSRLKQEEFFGRAMFMKIGDLKGMFGLLMVNMQMLRAKLKVLDISYGIGTANTALVYHHGKLLALSEADKPYAIKVLEDGDLQTIGLLDYDKRLAHSFTAHPKVDPFTGEMFTFGYSHTPPYVTYRVISKDGAMNDPVPITVSGPIMMHDFAITENYAIFMDLPLYFKPKEMVKDKKFIFSFDATQKARFGILPRYAKNELLIKWFELPNCFIFHNANAWEEGDEVVLITCRLENPDLDMVNSTVKERLDNFKNELYEMRFNLQNGLASQKKLSVSAVDFPRVNESYTTRKQRYVYGTTLDKIAKVTGIIKFDLHAEPETGKEKLELGGNVKGIFDLGPGRFGSEAVFVPRHPGITSEEDDGYLIFFVHDENTGKSAVNVIDAKTMSPDPVAVVELPKRVPYGFHAFFVTEDQLQEQAKV

SEQ ID NO: 51 - protein, 541 aa, Zea mays
MDSHRNDGVVVVPAPRPRKGLASWALDLLESLAVRLGHDKTKPLHWLSGNFAPVVEETPPAPNLSVRGHLPECLNGEFVRVGPNPKFAPVAGYHWFDGDGMIHAMRIKDGKATYVSRYVKTARLKQEEYFGGAKFMKIGDLKGFFGLFMVQMQQLRKKFKVLDFTYGFGTANTALIYHHGKLMALSEADKPYVVKVLEDGDLQTLGLLDYDKRLKHSFTAHPKVDPFTDEMFTFGYSHEPPYCTYRVINKEGAMLDPVPITIPESVMMHDFAITENYSIFMDLPLLFRPKEMVKNGEFIYKFDPTKKGRFGILPRYAKDDKLIRWFQLPNCFIFHNANAWEEGDEVVLITCRLENPDLDKVNGYQSDKLENFGNELYEMRFNMKTGAASQKQLSVSAVDFPRVNESYTGRKQRYVYCTILDSIAKVTGIIKFDLHAEPESGVKELEVGGNVQGIYDLGPGRFGSEAIFVPKHPGVSGEEDDGYLIFFVHDENTGKSEVNVIDAKTMSADPVAVVELPNRVPYGFHAFFVTEDQLARQAEGQ

SEQ ID NO: 52 - protein, 538 aa, Arabidopsis thaliana
MAEKLSDGSSIISVHPRPSKGFSSKLLDLLERLVVKLMHDASLPLHYLSGNFAPIRDETPPVKDLPVHGFLPECLNGEFVRVGPNPKFDAVAGYHWFDGDGMIHGVRIKDGKATYVSRYVKTSRLKQEEFFGAAKFMKIGDLKGFFGLLMVNVQQLRTKLKILDNTYGNGTANTALVYHHGKLLALQEADKPYVIKVLEDGDLQTLGIIDYDKRLTHSFTAHPKVDPVTGEMFTFGYSHTPPYLTYRVISKDGIMHDPVPITISEPIMMHDFAITETYAIFMDLPMHFRPKEMVKEKKMIYSFDPTKKARFGVLPRYAKDELMIRWFELPNCFIFHNANAWEEEDEVVLITCRLENPDLDMVSGKVKEKLENFGNELYEMRFNMKTGSASQKKLSASAVDFPRINECYTGKKQRYVYGTILDSIAKVTGIIKFDLHAEAETGKRMLEVGGNIKGIYDLGEGRYGSEAIYVPRETAEEDDGYLIFFVHDENTGKSCVTVIDAKTMSAEPVAVVELPHRVPYGFHALFVTEEQLQEQTLI

SEQ ID NO: 53 - protein, 545 aa, Solanum lycopersicum
MGRKEDDGVERIEGGVVVVNPKPRRGITAKAIDLLEWGIVKLMHDSSKPLHYLQGNFAPTDETPPLNDLVVQGHLPECLNGEFVRVGPNPKFAPVAGYHWFDGDGMIHGLRIKDGKATYVSRYVRTSRLKQEEFFGGAKFMKVGDLKGLFGLFTVYMQMLRTKLKVLDISYGNSTANTALVYHHGKLLALSEADKPYALKVLEDGDLQTLGMLDYDKRLTHSFTAHPKVDAVTGEMFTFGYAHTPPYITYRVISKDGIMQDPVPITIPEPIMMHDFAITENYAIMMDLPLCFRPKEMVKKNKLAFTFDATKKARFGVLPRYANNEALIRWFELPNCFIFHNANAWEEGDEVVLITCRLVNPDLDMVNGAVKEKLENFCNELYEMRFNMKSGAASQKKLSESAVDFPRINENYTGRKQRYVYGTTLNSIAKVTGVIKFDLHAEPETGKSQLEVGGNVQGIFDLGPGRFGSEAVFVPSRPGTEREEDDGYLIFFVHDENTGKSAVNVIDAKTMSAEPVAVVELPKRVPYGFHAFFVTEEQIQEQAKL

SEQ ID NO: 54 - protein, 599 aa, Chrysanthemum morifolium
MGSFPTSLLSTFLRPNSIPFQHQPPRRPLAPPTSLPQPSACRVFSTRIEENQPTVTTTRRPKRKWLKKLISSTRKHRSKSVKEDQPLPSMIFKVFDDIIINFIDPPLRVSVDPKYVLSHNFSPVNELPPTECEMIEGTLPSCLDGAYFRNGPNPQYLPRGPYHLFDGDGMLHAIRISKGKATFCSRYVKTYKYQTEKDAGSPIFPNVFSGFNGMTASIARLAVSTGRILMGQFDPTKGIGVANTSIAYFGNKLYALGESDLPYAIKLATNGDIITIGRDDFDGKLLTNMTAHPKIDPVTKETFAFRYGPGPPFLTFFWFNENGKKQDDVPIFSVISPSFIHDFAITKNYAIFPENQIEMSLTGLIGGGSPVRADPRKVARLGVIPRYDKDDSEMKWFEVPGLNVVHCINAWEEDHGDTIVMVAPNILSVEHALERMDLIHASVEKVTMDLKSGMVSRYPLSIRNLDFAVINPAFIAVKNRYIYCGVGDPMPKISGVVKLDISLSEVDRHECIVASRMFGRGCFGGEPFFVAKEPKNPYADEDDGYIVSYVHNEITGDSRFVVMDAKSPTLEIVAAVKLPHRVPYGFHGLFVRENDLTTL

SEQ ID NO: 55 - protein, 254 aa, Escherichia coli
MRSIARRTAVGAALLLVMPVAVWISGWRWQPGEQSWLLKAAFWVTETVTQPWGVITHLILFGWFLWCLRFRIKAAFVLFAILAAAILVGQGVKSWIKDKVQEPRPFVIWLEKTHHIPVDEFYTLKRAERGNLVKEQLAEEKNIPQYLRSHWQKETGFAFPSGHTMFAASWALLAVGLLWPRRRTLTIAILLVWATGVMGSRLLLGMHWPRDLVVATLISWALVAVATWLAQRICGPLTPPAEENREIAQREQES

SEQ ID NO: 56 - protein, 203 aa, Bacillus subtilis
MYKPVSLFLFFLILAAAIHTNAVQSADEAISKAAVLIRQPWLNEVMTGITHLGASSFLLPLIVIIGAGMFFYRKTWDGLLMLLVFGTDRLLNKVLKEWIERVRPDFAPLVHESSFSFPSGHSMNAACVYPVIAYFLVKHLPFLSKHKKMVYIIAGVIAVLVGISRVYLGVHFVTDVLGGFSLGLLLFFLVKGFDEKIKRFRQK

SEQ ID NO: 57 - protein, 647 aa, Escherichia coli
MIKFSATLLATLIAASVNAATVDLRIMETTDLHSNMMDFDYYKDTATEKFGLVRTASLINDARNEVKNSVLVDNGDLIQGSPLADYMSAKGLKAGDIHPVYKALNTLDYTVGTLGNHEFNYGLDYLKNALAGAKFPYVNANVIDARTKQPMFTPYLIKDTEVVDKDGKKQTLKIGYIGVVPPQIMGWDKANLSGKVTVNDITETVRKYVPEMREKGADVVVVLAHSGLSADPYKVMAENSVYYLSEIPGVNAIMFGHAHAVFPGKDFADIEGADIAKGTLNGVPAVMPGMWGDHLGVVDLQLSNDSGKWQVTQAKAEARPIYDIANKKSLAAEDSKLVETLKADHDATRQFVSKPIGKSADNMYSYLALVQDDPTVQVVNNAQKAYVEHYIQGDPDLAKLPVLSAAAPFKVGGRKNDPASYVEVEKGQLTFRNAADLYLYPNTLIVVKASGKEVKEWLECSAGQFNQIDPNSTKPQSLINWDGFRTYNFDVIDGVNYQIDVTQPARYDGECQMINANAERIKNLTFNGKPIDPNAMFLVATNNYRAYGGKFAGTGDSHIAFASPDENRSVLAAWIADESKRAGEIHPAADNNWRLAPIAGDKKLDIRFETSPSDKAAAFIKEKGQYPMNKVATDDIGFAIYQVDLSK

SEQ ID NO: 58 - protein, 647 aa, Salmonella typhimurium
MIKFSATLLATLIAASVNAATVDLRIMETTDLHSNMMDFDYYKDTATEKFGLVRTASLIHAARNEVKNSVLVDNGDLIQGSPLGDYMAAKGLKDGDVHPVYKALNTLDYAVGNLGNHEFNYGLDYLHNALAGAKFPYVNANIIDVKTQKPLFTPYLIKETSVIDKDGNPQTLKIGYIGFVPPQIMIWDKANLSGKVTVNDITETARKYVPEMREKGADIVVVIAHSGLSADPYHSMAENSVYYLSEVPGVDAIMFGHAHAVFPGKDFADIKGADIAKGTLNGIPAVMPGMWGDHLGVVDLVLNNDSGKWQVTQAKAEARPIYDAAAKKSLAAEDSKLVGILKADHDATREFVSKPIGKSADNMYSYLALVQDDPTVQVVNNAQKAYVEHFIQGDPDLAKLPVLSAAAPFKVGGRKNDPASFVEVEKGQLTFRNAADLYLYPNTLVVVKASGKEVKEWLECSAGQFNQIDIHSNKPQSLINWDGFRTYNFDVIDGVNYQIDVSQPARYDGECQMVNPQAERIKNLTFNGKPVDPNATFLVATNNYRAYGGKFAGTGDSHIAFASPDENRAVLAAWIGAESKRAGEIHPAADNNWRLAPIHSDTALDIRFETSPGDKAAAFIKAKGQYPMKKVAVDDIGFAIYQVDLSK

SEQ ID NO: 59 - protein, 105 aa, Escherichia coli
MAEWSGEYISPYAEHGKKSEQVKKITVSIPLKVLKILTDERTRRQVNNLRHATNSELLCEAFLHAFTGQPLPDDADLRKERSDEIPEAAKEIMREMGINPETWEY

SEQ ID NO: 60 - protein, 105 aa, Salmonella typhimurium
MAEWSGEYISPYAEHGKKSEQVKKITVSIPLKVLKILTDERTRRQVNNLRHATNSELLCEAFLHAFTGQPLPDDADLRKERSDEIPEAAKEIMRELGIDPETWEY